European Patent Specification EP 3 715 459 B1, published April 24, 2024. Title: H9 AVIAN INFLUENZA VACCINE STRAIN WHICH DIFFERENTIATES INFECTED FROM VACCINATED ANIMALS, AND PREPARATION METHOD THEREFOR. Applicant: Song, Jiasheng. Application PCT/CN2018/089527. The sequence listing filed with the application follows.

SEQUENCE LISTING (8 sequences)

SEQ ID NO: 1 - DNA, 1743 bp, artificial sequence
  the DNA sequence of HA gene
agcaaaagcaggggaatttcacaaccactcaagatggatacagcatcactgataactatactactagtaataacagtaagcaatgcagataagatctgcatcggctatcaatcaacgaactccacagaaactgtagacacactaacagaaaacaatgtccctgtgacacatgccaaagaactgctccacacagagcataatgggatgctgtgtgcaacaagcttgggacaccctcttattctagacacctgtactattgaaggactaatctatggcaatccctcttgtgatctattcttgggaggaagagaatggtcctatatcgtcgagagaccatcagctgtcaacggattgtgttatcccgggaatgtagaaaatctggaagagctaaggtcactttttagttctgctaggtcttatcaaaggatccagattttcccagacacaatctggaatgtgtcttacagtgggacaagcaaagcatgttcagattcattctacagaagcatgagatggttgactcaaaagaacaacgcttaccctattcaagacgcccaatacacaaataatcaagaaaagaacattcttttcatgtggggcataaatcacccacccaccgatactgcgcaaacaaatctgtacacaagaaccgacacaacaacgagtgtggcaacagaagaaataaacaggaccttcaaaccattgataggaccaaggcctcttgttaacggtttgatgggaaggattaattattattggtctgtattgaaaccgggtcaaacactgcgaataaaatctaatggaaatctaatagctccgtggtatggacacattctctcaggggagagccacggaagaatcctgaagactgatttaaaaaggggtagctgcacagtacaatgtcagacagagaagggtggcttaaacacaacattgccattccaaaatgtgagtaagtatgcatttggaaactgctcaaaatacattggcataaagagtctcaaacttgcagttggtctgaggaatgtaccttctagatctagtagaggactattcggggccatagcaggattcatagaaggaggttggtcagggctagttgctggttggtatggattccagcattcaaatgaccaaggggttggtatggcagcggatagagactcaacccaaaaggcaattgataaaataacatccaaagtgaataacatagtcgacaaaatgaacaagcagtatgaaattatcgatcatgagttcagcgaggttgaaactagacttaacatgatcaacaataagattgatgatcaaatccaagatatatgggcatataatgcagaattgctagttctgcttgaaaaccagaaaacactcgatgaacatgatgcaaatgtaaacaatctatataataaagtgaaaagggcattgggttccaatgcggtggaagatgggaaaggatgtttcgagttataccacaaatgtgatgaccagtgcatggagacaattcgaaacgggacctacaacagaaggaagtatcaagaggagtcaaaattagaaagacagaaaatagagggggtcaagctggaatctgaaggaacttacaaaatcctcaccatttattcgactgtcgcctcatctcttgtaattgcaatggggtttgctgccttcttgttctgggccatgtccaatgggtcttgcagatgcaacatttgtatataattggcaaaaacaccctttgtttctact

SEQ ID NO: 2 - protein, 560 aa, artificial sequence
  the amino acid sequence encoded by the H9 subtype HA gene
MDTASLITILLVITVSNADKICIGYQSTNSTETVDTLTENNVPVTHAKELLHTEHNGMLCATSLGHPLILDTCTIEGLIYGNPSCDLFLGGREWSYIVERPSAVNGLCYPGNVENLEELRSLFSSARSYQRIQIFPDTIWNVSYSGTSKACSDSFYRSMRWLTQKNNAYPIQDAQYTNNQEKNILFMWGINHPPTDTAQTNLYTRTDTTTSVATEEINRTFKPLIGPRPLVNGLMGRINYYWSVLKPGQTLRIKSNGNLIAPWYGHILSGESHGRILKTDLKRGSCTVQCQTEKGGLNTTLPFQNVSKYAFGNCSKYIGIKSLKLAVGLRNVPSRSSRGLFGAIAGFIEGGWSGLVAGWYGFQHSNDQGVGMAADRDSTQKAIDKITSKVNNIVDKMNKQYEIIDHEFSEVETRLNMINNKIDDQIQDIWAYNAELLVLLENQKTLDEHDANVNNLYNKVKRALGSNAVEDGKGCFELYHKCDDQCMETIRNGTYNRRKYQEESKLERQKIEGVKLESEGTYKILTIYSTVASSLVIAMGFAAFLFWAMSNGSCRCNICI

SEQ ID NO: 3 - DNA, 203 bp, artificial sequence
  5'-end packaging signal sequence
agcaaaagcaggggtttaaaatgaatccaaatcagaaaataataaccattggatcaatctgtctggtagtcggactaattagcctaatattgcaaatagggaatataatctcaatatggattagccattcaattcaaactggaagtcaaaaccatactggaatatgcaaccaaaacatcattacctataaaaatagcacctgg

SEQ ID NO: 4 - DNA, 185 bp, artificial sequence
  3'-end packaging signal sequence
gaggccgtgcttctgggttgaattaatcaggggacgacctaaagaaaaaacaatctggactagtgcgagcagcatttctttttgtggcgtgaatagtgatactgtagattggtcttggccagacggtgctgagttgccattcagcattgacaagtagtctgttcaaaaaactccttgtttctact

SEQ ID NO: 5 - DNA, 1224 bp, artificial sequence
  the sequence containing type B NA extracellular region
gttcaggctgtaaatcattctgcagcaaaaggggtgacacttcttctcccagaaccggaatggacataccctcgtttatcttgcccgggctcaacctttcagaaagcactcctaattagcccccatagattcggagaaatcaaaggaaactcagctcccttgataataagggaaccttttattgcttgtggaccaacggaatgcaaacactttgctctaacccattatgcagctcaaccagggggatactacaatggaacaagagaagacagaaacaagctgaggcatctaatttcagtcaaattgggcaaaatcccaacagtagaaaactccattttccacatggcagcttggagcgggtccgcatgccatgatggtaaagaatggacatatatcggagttgatggccccgacagtaatgcattgctcaaaataaaatatggagaagcatatactgacacataccattcctatgcaaaaaacatcctaaggacacaagaaagtgcctgcaattgcatcgggggagattgttatcttatgataactgatggcccagcttcaggggttagtgaatgcagattccttaagattcgagagggcagaataataaaagaaatatttccaacaggaagagtaaaacatactgaggaatgcacatgcggatttgccagcaacaaaaccatagaatgtgcttgtagagataaccgttacacagcaaaaagaccctttgtcaaattaaatgtggagactgatacagcggaaataagattgatgtgcacagagacttatttggacacccccagaccaaatgatggaagcataacagggccttgcgaatctgatggggacaaagggagtggaggcatcaagggaggatttgttcatcaaagaatggcatccaagattggaaggtggtactctcgaacgatgtctaaaaccaaaagaatggggatgggactgtatgtaaaatatgatggagacccatggactgacagtgaagcccttgctcttagtggagtaatggtttcaatggaagaacctggttggtattcctttggcttcgaaataaaagataagaaatgtgatgtcccctgtattgggatagaaatggtacatgatggtgggaaaacgacttggcactcagcagcaacagccatttattgtttaatgggctcaggacaattgctgtgggacactgtcacaggtgttgatatggctctgtaa

SEQ ID NO: 6 - DNA, 1224 bp, artificial sequence
  the DNA sequence for coding the extracellular region protein amino acid sequence in influenza B virus NA
gttcaggctgtgaaccgttctgcaacaaaaggggtgacacttcttctcccagaaccggagtggacatacccgcgtttatcttgcccgggctcaacctttcagaaagcactcctaattagccctcatagattcggagaaaccaaaggaaactcagctcccttgataataagggaaccttttattgcttgtggaccaaatgaatgcaaacactttgctctaacccattatgcagcccaaccagggggatactacaatggaacaagaggagacagaaacaagctgaggcatctaatttcagtcaaattgggcaaaatcccaacagtagaaaactccattttccacatggcagcatggagcgggtccgcgtgccatgatggtaaggaatggacatatatcggagttgatggccctgacaataatgcattgctcaaagtaaaatatggagaagcatatactgacacataccattcctatgcaaacaaaatcctaagaacacaagaaagtgcctgcaattgcatcgggggaaattgttatcttatgataactgatggctcagcttcaggtgttagtgaatgcagatttcttaagattcgagagggccgaataataaaagaaatatttccaacaggaagagtaaaacacactgaggaatgcacatgcggatttgccagcaataaaaccatagaatgtgcctgtagagataacagttacacagcaaaaagaccttttgtcaaattaaacgtggagactgatacagcagaaataagattgatgtgcacagatacttatttggacacccccagaccaaacgatggaagcataacaggcccttgtgaatctaatggggacaaagggagtggaggcatcaagggaggatttgttcatcaaagaatggaatccaagattggaaggtggtactctcgaacgatgtctaaaactgaaaggatggggatgggactgtatgtcaagtatgatggagacccatgggctgacagtgatgccctagcttttagtggagtaatggtttcaatgaaagaacctggttggtactcctttggcttcgaaataaaagataagaaatgcgatgtcccctgtattgggatagagatggtacatgatggtggaaaagagacttggcactcagcagcaacagccatttactgtttaatgggctcaggacagctgctgtgggacactgtcacaggtgttgacatggctctgtaa

SEQ ID NO: 7 - DNA, 36 bp, artificial sequence
  Up-primer
cacacacgtctccgggagcaaaagcaggggaatttc

SEQ ID NO: 8 - DNA, 41 bp, artificial sequence
  Low-Primer
cacacacgtctcctattagtagaaacaaagggtgtttttgc